European Patent Application EP 4 137 510 A1, published February 22, 2023. Title: PD-1 mutant polypeptide and preparation and application thereof. Applicant: NANTONG YICHEN BIOPHARMA.CO.LTD. The sequence listing filed with the application follows.

SEQUENCE LISTING (100 sequences)

SEQ ID NO: 1 - DNA, 429 bp, Artificial Sequence
  Synthesized
ctggacagcccagataggccatggaacccacctactttctctcctgcactgctggtggttacagaaggagataatgctacctttacttgctccttttccaacactagtgagagttttgtccttaattggtatagaatgtctccttcaaatcagacggacaagctcgctgcatttcctgaggaccgcagtcagccggggcaagattccagattccgcgtgacccagctccccaacggacgcgattttcacatgtccgttgtcagggcacgacgcaacgatagtgggacttatctgtgcggggcgatcagtctggccccgaaggtccagataaaagagtccctccgcgctgaactcagggtgaccgagagacgggccgaagtgcccacagcacacccaagtccaagcccaagacctgctgggcaattccaa

SEQ ID NO: 2 - protein, 143 aa, Artificial Sequence
  Synthesized
LDSPDRPWNPPTFSPALLVVTEGDNATFTCSFSNTSESFVLNWYRMSPSNQTDKLAAFPEDRSQPGQDSRFRVTQLPNGRDFHMSVVRARRNDSGTYLCGAISLAPKVQIKESLRAELRVTERRAEVPTAHPSPSPRPAGQFQ

SEQ ID NO: 3 - DNA, 1344 bp, Artificial Sequence
  Synthesized
caggtgcagctgcaggagagcggccccggcctggtgaagcccagcgagaccctgagcctgacctgcaccgtgagcggcggcagcgtgagcagcggcgactactactggacctggatccgccagagccccggcaagggcctggagtggatcggccacatctactacagcggcaacaccaactacaaccccagcctgaagagccgcctgaccatcagcatcgacaccagcaagacccagttcagcctgaagctgagcagcgtgaccgccgccgacaccgccatctactactgcgtgcgcgaccgcgtgaccggcgccttcgacatctggggccagggcaccatggtgactgtgtctagcgcctccaccaagggcccatcggtcttccccctggcaccctcctccaagagcacctctgggggcacagcggccctgggctgcctggtcaaggactacttccccgaaccggtgacggtgtcgtggaactcaggcgccctgaccagcggcgtgcacaccttcccggctgtcctacagtcctcaggactctactccctcagcagcgtggtgactgtgccctctagcagcttgggcacccagacctacatctgcaacgtgaatcacaagcccagcaacaccaaggtggacaagaaagttgaacccaaatcttgcgacaaaactcacacatgcccaccgtgcccagcacctccagtcgccggaccgtcagtcttcctcttccctccaaaacccaaggacaccctcatgatctcccggacccctgaggtcacatgcgtggtggtggacgtgagccacgaagaccctgaggtcaagttcaactggtacgtggacggcgtggaggtgcataatgccaagacaaagccgcgggaggagcagtacaacagcacgtaccgtgtggtcagcgtcctcaccgtcctgcaccaggactggctgaatggcaaggagtacaagtgcaaggtctccaacaaaggcctcccaagctccatcgagaaaaccatctccaaagccaaagggcagccccgagaaccacaggtgtacaccctgcctccatcccgggatgagctgaccaagaaccaggtcagcctgacctgcctggtcaaaggcttctatcccagcgacatcgccgtggagtgggagagcaatgggcagccggagaacaactacaagaccacgcctcccgtgctggactccgacggctccttcttcctctacagcaagctcaccgtggacaagagcaggtggcagcaggggaacgtcttctcatgctccgtgatgcatgaggctctgcacaaccactacacgcagaagagcctctccctgtctccgggtaaa

SEQ ID NO: 4 - protein, 448 aa, Artificial Sequence
  Synthesized
QVQLQESGPGLVKPSETLSLTCTVSGGSVSSGDYYWTWIRQSPGKGLEWIGHIYYSGNTNYNPSLKSRLTISIDTSKTQFSLKLSSVTAADTAIYYCVRDRVTGAFDIWGQGTMVTVSSASTKGPSVFPLAPSSKSTSGGTAALGCLVKDYFPEPVTVSWNSGALTSGVHTFPAVLQSSGLYSLSSVVTVPSSSLGTQTYICNVNHKPSNTKVDKKVEPKSCDKTHTCPPCPAPPVAGPSVFLFPPKPKDTLMISRTPEVTCVVVDVSHEDPEVKFNWYVDGVEVHNAKTKPREEQYNSTYRVVSVLTVLHQDWLNGKEYKCKVSNKGLPSSIEKTISKAKGQPREPQVYTLPPSRDELTKNQVSLTCLVKGFYPSDIAVEWESNGQPENNYKTTPPVLDSDGSFFLYSKLTVDKSRWQQGNVFSCSVMHEALHNHYTQKSLSLSPGK

SEQ ID NO: 5 - DNA, 642 bp, Artificial Sequence
  Synthesized
gacatccagatgacccagagccccagcagcctgagcgccagcgtgggcgaccgcgtgaccatcacctgccaggccagccaggacatcagcaactacctgaactggtaccagcagaagcccggcaaggcccccaagctgctgatctacgacgccagcaacctggagaccggcgtgcccagccgcttcagcggcagcggcagcggcaccgacttcaccttcaccatcagcagcctgcagcccgaggacatcgccacctacttctgccagcacttcgaccacctgcccctggccttcggcggcggcaccaaggtggagatcaagcgcacagtggcagcccccagcgtcttcatttttcccccttccgatgaacagctgaagtccggcactgcttctgtggtctgtctgctgaacaatttctatcccagagaggccaaggtgcagtggaaagtggacaacgctctgcagtccggcaacagccaggagagtgtgaccgaacaggatagtaaggacagcacatattctctgtctagtaccctgacactgagtaaggcagattacgagaagcacaaagtgtatgcctgcgaagtcactcatcagggactgtcaagccccgtgaccaagagcttcaaccggggcgagtgt

SEQ ID NO: 6 - protein, 214 aa, Artificial Sequence
  Synthesized
DIQMTQSPSSLSASVGDRVTITCQASQDISNYLNWYQQKPGKAPKLLIYDASNLETGVPSRFSGSGSGTDFTFTISSLQPEDIATYFCQHFDHLPLAFGGGTKVEIKRTVAAPSVFIFPPSDEQLKSGTASVVCLLNNFYPREAKVQWKVDNALQSGNSQESVTEQDSKDSTYSLSSTLTLSKADYEKHKVYACEVTHQGLSSPVTKSFNRGEC

SEQ ID NO: 7 - DNA, 642 bp, Artificial Sequence
  Synthesized
gacatccagatgacccagtctccatcctccctgtctgcatctgtaggagacagagtcaccatcacttgccgggcaagtcaggatgtgaataccgcggtcgcatggtatcagcagaaaccagggaaagcccctaagctcctgatctattctgcatccttcttgtatagtggggtcccatcaaggttcagtggcagtagatctgggacagatttcactctcaccatcagcagtctgcaacctgaagattttgcaacttactactgtcaacagcattacactacccctccgacgttcggccaaggtaccaaggtggagatcaaacgaactgtggctgcaccatctgtcttcatcttcccgccatctgatgagcagttgaaatctggaactgcctctgtcgtgtgcctgctgaataacttctatcccagagaggccaaagtacagtggaaggtggataacgccctccaatcgggtaactcccaggagagtgtcacagagcaggacagcaaggacagcacctacagcctcagcagcaccctgacgctgagcaaagcagactacgagaaacacaaagtctacgcctgcgaagtcacccatcagggcctgtcctcgcccgtcacaaagagcttcaacaggggagagtgt

SEQ ID NO: 8 - protein, 214 aa, Artificial Sequence
  Synthesized
DIQMTQSPSSLSASVGDRVTITCRASQDVNTAVAWYQQKPGKAPKLLIYSASFLYSGVPSRFSGSRSGTDFTLTISSLQPEDFATYYCQQHYTTPPTFGQGTKVEIKRTVAAPSVFIFPPSDEQLKSGTASVVCLLNNFYPREAKVQWKVDNALQSGNSQESVTEQDSKDSTYSLSSTLTLSKADYEKHKVYACEVTHQGLSSPVTKSFNRGEC

SEQ ID NO: 9 - DNA, 1347 bp, Artificial Sequence
  Synthesized
gaggtgcagctggtggagtctggaggaggcttggtccagcctggggggtccctgagactctcctgtgcagcctctgggttcaatattaaggacacttacatccactgggtccgccaggctccagggaaggggctggagtgggtcgcacgtatttatcctaccaatggttacacacgctacgcagactccgtgaagggccgattcaccatctccgcagacacttccaagaacacggcgtatcttcaaatgaacagcctgagagccgaggacacggccgtgtattactgttcgagatggggcggtgacggcttctatgccatggactactggggccaaggaaccctggtcaccgtctcctcagcctccaccaagggcccatcggtcttccccctggcaccctcctccaagagcacctctgggggcacagcggccctgggctgcctggtcaaggactacttccccgaaccggtgacggtgtcgtggaactcaggcgccctgaccagcggcgtgcacaccttcccggctgtcctacagtcctcaggactctactccctcagcagcgtggtgactgtgccctctagcagcttgggcacccagacctacatctgcaacgtgaatcacaagcccagcaacaccaaggtggacaagaaagttgaacccaaatcttgcgacaaaactcacacatgcccaccgtgcccagcacctccagtcgccggaccgtcagtcttcctcttccctccaaaacccaaggacaccctcatgatctcccggacccctgaggtcacatgcgtggtggtggacgtgagccacgaagaccctgaggtcaagttcaactggtacgtggacggcgtggaggtgcataatgccaagacaaagccgcgggaggagcagtacaacagcacgtaccgtgtggtcagcgtcctcaccgtcctgcaccaggactggctgaatggcaaggagtacaagtgcaaggtctccaacaaaggcctcccaagctccatcgagaaaaccatctccaaagccaaagggcagccccgagaaccacaggtgtacaccctgcctccatcccgggatgagctgaccaagaaccaggtcagcctgacctgcctggtcaaaggcttctatcccagcgacatcgccgtggagtgggagagcaatgggcagccggagaacaactacaagaccacgcctcccgtgctggactccgacggctccttcttcctctacagcaagctcaccgtggacaagagcaggtggcagcaggggaacgtcttctcatgctccgtgatgcatgaggctctgcacaaccactacacgcagaagagcctctccctgtctccgggtaaa

SEQ ID NO: 10 - protein, 449 aa, Artificial Sequence
  Synthesized
EVQLVESGGGLVQPGGSLRLSCAASGFNIKDTYIHWVRQAPGKGLEWVARIYPTNGYTRYADSVKGRFTISADTSKNTAYLQMNSLRAEDTAVYYCSRWGGDGFYAMDYWGQGTLVTVSSASTKGPSVFPLAPSSKSTSGGTAALGCLVKDYFPEPVTVSWNSGALTSGVHTFPAVLQSSGLYSLSSVVTVPSSSLGTQTYICNVNHKPSNTKVDKKVEPKSCDKTHTCPPCPAPPVAGPSVFLFPPKPKDTLMISRTPEVTCVVVDVSHEDPEVKFNWYVDGVEVHNAKTKPREEQYNSTYRVVSVLTVLHQDWLNGKEYKCKVSNKGLPSSIEKTISKAKGQPREPQVYTLPPSRDELTKNQVSLTCLVKGFYPSDIAVEWESNGQPENNYKTTPPVLDSDGSFFLYSKLTVDKSRWQQGNVFSCSVMHEALHNHYTQKSLSLSPGK

SEQ ID NO: 11 - DNA, 429 bp, Artificial Sequence
  Synthesized
ctggacagcccagataggccatggaacccacctactttctctcctgcactgctggtggttacagaaggagataatgctacctttacttgctccttttccaacactagtgagagttttgtccttaattggtatagaatgtctccttcaaatcagacggacaagctcgctgcatttcctgaggaccgcagtcagccggggcaagattgcagattccgcgtgacccagctccccaacggacgcgattttcacatgtccgttgtcagggcacgacgcaacgatagtgggacttatctgtgcggggcgatcagtctggccccgaaggcccagataaaagagtccctccgcgctgaactcagggtgaccgagagacgggccgaagtgcccacagcacacccaagtccaagcccaagacctgctgggcaattccaa

SEQ ID NO: 12 - protein, 143 aa, Artificial Sequence
  Synthesized
LDSPDRPWNPPTFSPALLVVTEGDNATFTCSFSNTSESFVLNWYRMSPSNQTDKLAAFPEDRSQPGQDCRFRVTQLPNGRDFHMSVVRARRNDSGTYLCGAISLAPKAQIKESLRAELRVTERRAEVPTAHPSPSPRPAGQFQ

SEQ ID NO: 13 - protein, 7 aa, Artificial Sequence
  Synthesized
SGDYYWT

SEQ ID NO: 14 - protein, 16 aa, Artificial Sequence
  Synthesized
HIYYSGNTNYNPSLKS

SEQ ID NO: 15 - protein, 8 aa, Artificial Sequence
  Synthesized
DRVTGAFD

SEQ ID NO: 16 - protein, 11 aa, Artificial Sequence
  Synthesized
QASQDISNYLN

SEQ ID NO: 17 - protein, 7 aa, Artificial Sequence
  Synthesized
DASNLET

SEQ ID NO: 18 - protein, 9 aa, Artificial Sequence
  Synthesized
QHFDHLPLA

SEQ ID NO: 19 - protein, 5 aa, Artificial Sequence
  Synthesized
DTYIH

SEQ ID NO: 20 - protein, 17 aa, Artificial Sequence
  Synthesized
RIYPTNGYTRYADSVKG

SEQ ID NO: 21 - protein, 11 aa, Artificial Sequence
  Synthesized
WGGDGFYAMDY

SEQ ID NO: 22 - protein, 11 aa, Artificial Sequence
  Synthesized
RASQDVNTAVA

SEQ ID NO: 23 - protein, 7 aa, Artificial Sequence
  Synthesized
SASFLYS

SEQ ID NO: 24 - protein, 14 aa, Artificial Sequence
  Synthesized
QQHYTTPPTFGQGT

SEQ ID NO: 25 - DNA, 1119 bp, Artificial Sequence
  Synthesized
ctggacagcccagataggccatggaacccacctactttctctcctgcactgctggtggttacagaaggagataatgctacctttacttgctccttttccaacactagtgagagttttgtccttaattggtatagaatgtctccttcaaatcagacggacaagctcgctgcatttcctgaggaccgcagtcagccggggcaagattgcagattccgcgtgacccagctccccaacggacgcgattttcacatgtccgttgtcagggcacgacgcaacgatagtgggacttatctgtgcggggcgatcagtctggccccgaaggcccagataaaagagtccctccgcgctgaactcagggtgaccgagagacgggccgaagtgcccacagcacacccaagtccaagcccaagacctgctgggcaattccaaggcggaggcggatccggaggcggaggttccggcgggggtgggagcggggacatccagatgacccagagccccagcagcctgagcgccagcgtgggcgaccgcgtgaccatcacctgccaggccagccaggacatcagcaactacctgaactggtaccagcagaagcccggcaaggcccccaagctgctgatctacgacgccagcaacctggagaccggcgtgcccagccgcttcagcggcagcggcagcggcaccgacttcaccttcaccatcagcagcctgcagcccgaggacatcgccacctacttctgccagcacttcgaccacctgcccctggccttcggcggcggcaccaaggtggagatcaagcgcacagtggcagcccccagcgtcttcatttttcccccttccgatgaacagctgaagtccggcactgcttctgtggtctgtctgctgaacaatttctatcccagagaggccaaggtgcagtggaaagtggacaacgctctgcagtccggcaacagccaggagagtgtgaccgaacaggatagtaaggacagcacatattctctgtctagtaccctgacactgagtaaggcagattacgagaagcacaaagtgtatgcctgcgaagtcactcatcagggactgtcaagccccgtgaccaagagcttcaaccggggcgagtgt

SEQ ID NO: 26 - protein, 373 aa, Artificial Sequence
  Synthesized
LDSPDRPWNPPTFSPALLVVTEGDNATFTCSFSNTSESFVLNWYRMSPSNQTDKLAAFPEDRSQPGQDCRFRVTQLPNGRDFHMSVVRARRNDSGTYLCGAISLAPKAQIKESLRAELRVTERRAEVPTAHPSPSPRPAGQFQGGGGSGGGGSGGGGSGDIQMTQSPSSLSASVGDRVTITCQASQDISNYLNWYQQKPGKAPKLLIYDASNLETGVPSRFSGSGSGTDFTFTISSLQPEDIATYFCQHFDHLPLAFGGGTKVEIKRTVAAPSVFIFPPSDEQLKSGTASVVCLLNNFYPREAKVQWKVDNALQSGNSQESVTEQDSKDSTYSLSSTLTLSKADYEKHKVYACEVTHQGLSSPVTKSFNRGEC

SEQ ID NO: 27 - DNA, 1119 bp, Artificial Sequence
  Synthesized
ctggacagcccagataggccatggaacccacctactttctctcctgcactgctggtggttacagaaggagataatgctacctttacttgctccttttccaacactagtgagagttttgtccttaattggtatagaatgtctccttcaaatcagacggacaagctcgctgcatttcctgaggaccgcagtcagccggggcaagattccagattccgcgtgacccagctccccaacggacgcgattttcacatgtccgttgtcagggcacgacgcaacgatagtgggacttatctgtgcggggcgatcagtctggccccgaaggtccagataaaagagtccctccgcgctgaactcagggtgaccgagagacgggccgaagtgcccacagcacacccaagtccaagcccaagacctgctgggcaattccaaggcggaggcggatccggaggcggaggttccggcgggggtgggagcggggacatccagatgacccagagccccagcagcctgagcgccagcgtgggcgaccgcgtgaccatcacctgccaggccagccaggacatcagcaactacctgaactggtaccagcagaagcccggcaaggcccccaagctgctgatctacgacgccagcaacctggagaccggcgtgcccagccgcttcagcggcagcggcagcggcaccgacttcaccttcaccatcagcagcctgcagcccgaggacatcgccacctacttctgccagcacttcgaccacctgcccctggccttcggcggcggcaccaaggtggagatcaagcgcacagtggcagcccccagcgtcttcatttttcccccttccgatgaacagctgaagtccggcactgcttctgtggtctgtctgctgaacaatttctatcccagagaggccaaggtgcagtggaaagtggacaacgctctgcagtccggcaacagccaggagagtgtgaccgaacaggatagtaaggacagcacatattctctgtctagtaccctgacactgagtaaggcagattacgagaagcacaaagtgtatgcctgcgaagtcactcatcagggactgtcaagccccgtgaccaagagcttcaaccggggcgagtgt

SEQ ID NO: 28 - protein, 373 aa, Artificial Sequence
  Synthesized
LDSPDRPWNPPTFSPALLVVTEGDNATFTCSFSNTSESFVLNWYRMSPSNQTDKLAAFPEDRSQPGQDSRFRVTQLPNGRDFHMSVVRARRNDSGTYLCGAISLAPKVQIKESLRAELRVTERRAEVPTAHPSPSPRPAGQFQGGGGSGGGGSGGGGSGDIQMTQSPSSLSASVGDRVTITCQASQDISNYLNWYQQKPGKAPKLLIYDASNLETGVPSRFSGSGSGTDFTFTISSLQPEDIATYFCQHFDHLPLAFGGGTKVEIKRTVAAPSVFIFPPSDEQLKSGTASVVCLLNNFYPREAKVQWKVDNALQSGNSQESVTEQDSKDSTYSLSSTLTLSKADYEKHKVYACEVTHQGLSSPVTKSFNRGEC

SEQ ID NO: 29 - DNA, 1119 bp, Artificial Sequence
  Synthesized
ctggacagcccagataggccatggaacccacctactttctctcctgcactgctggtggttacagaaggagataatgctacctttacttgctccttttccaacactagtgagagttttgtccttaattggtatagaatgtctccttcaaatcagacggacaagctcgctgcatttcctgaggaccgcagtcagccggggcaagattgcagattccgcgtgacccagctccccaacggacgcgattttcacatgtccgttgtcagggcacgacgcaacgatagtgggacttatctgtgcggggcgatcagtctggccccgaaggcccagataaaagagtccctccgcgctgaactcagggtgaccgagagacgggccgaagtgcccacagcacacccaagtccaagcccaagacctgctgggcaattccaaggcggaggcggatccggaggcggaggttccggcgggggtgggagcggggacatccagatgacccagtctccatcctccctgtctgcatctgtaggagacagagtcaccatcacttgccgggcaagtcaggatgtgaataccgcggtcgcatggtatcagcagaaaccagggaaagcccctaagctcctgatctattctgcatccttcttgtatagtggggtcccatcaaggttcagtggcagtagatctgggacagatttcactctcaccatcagcagtctgcaacctgaagattttgcaacttactactgtcaacagcattacactacccctccgacgttcggccaaggtaccaaggtggagatcaaacgaactgtggctgcaccatctgtcttcatcttcccgccatctgatgagcagttgaaatctggaactgcctctgtcgtgtgcctgctgaataacttctatcccagagaggccaaagtacagtggaaggtggataacgccctccaatcgggtaactcccaggagagtgtcacagagcaggacagcaaggacagcacctacagcctcagcagcaccctgacgctgagcaaagcagactacgagaaacacaaagtctacgcctgcgaagtcacccatcagggcctgtcctcgcccgtcacaaagagcttcaacaggggagagtgt

SEQ ID NO: 30 - protein, 373 aa, Artificial Sequence
  Synthesized
LDSPDRPWNPPTFSPALLVVTEGDNATFTCSFSNTSESFVLNWYRMSPSNQTDKLAAFPEDRSQPGQDCRFRVTQLPNGRDFHMSVVRARRNDSGTYLCGAISLAPKAQIKESLRAELRVTERRAEVPTAHPSPSPRPAGQFQGGGGSGGGGSGGGGSGDIQMTQSPSSLSASVGDRVTITCRASQDVNTAVAWYQQKPGKAPKLLIYSASFLYSGVPSRFSGSRSGTDFTLTISSLQPEDFATYYCQQHYTTPPTFGQGTKVEIKRTVAAPSVFIFPPSDEQLKSGTASVVCLLNNFYPREAKVQWKVDNALQSGNSQESVTEQDSKDSTYSLSSTLTLSKADYEKHKVYACEVTHQGLSSPVTKSFNRGEC

SEQ ID NO: 31 - DNA, 1119 bp, Artificial Sequence
  Synthesized
ctggacagcccagataggccatggaacccacctactttctctcctgcactgctggtggttacagaaggagataatgctacctttacttgctccttttccaacactagtgagagttttgtccttaattggtatagaatgtctccttcaaatcagacggacaagctcgctgcatttcctgaggaccgcagtcagccggggcaagattccagattccgcgtgacccagctccccaacggacgcgattttcacatgtccgttgtcagggcacgacgcaacgatagtgggacttatctgtgcggggcgatcagtctggccccgaaggtccagataaaagagtccctccgcgctgaactcagggtgaccgagagacgggccgaagtgcccacagcacacccaagtccaagcccaagacctgctgggcaattccaaggcggaggcggatccggaggcggaggttccggcgggggtgggagcggggacatccagatgacccagtctccatcctccctgtctgcatctgtaggagacagagtcaccatcacttgccgggcaagtcaggatgtgaataccgcggtcgcatggtatcagcagaaaccagggaaagcccctaagctcctgatctattctgcatccttcttgtatagtggggtcccatcaaggttcagtggcagtagatctgggacagatttcactctcaccatcagcagtctgcaacctgaagattttgcaacttactactgtcaacagcattacactacccctccgacgttcggccaaggtaccaaggtggagatcaaacgaactgtggctgcaccatctgtcttcatcttcccgccatctgatgagcagttgaaatctggaactgcctctgtcgtgtgcctgctgaataacttctatcccagagaggccaaagtacagtggaaggtggataacgccctccaatcgggtaactcccaggagagtgtcacagagcaggacagcaaggacagcacctacagcctcagcagcaccctgacgctgagcaaagcagactacgagaaacacaaagtctacgcctgcgaagtcacccatcagggcctgtcctcgcccgtcacaaagagcttcaacaggggagagtgt

SEQ ID NO: 32 - protein, 373 aa, Artificial Sequence
  Synthesized
LDSPDRPWNPPTFSPALLVVTEGDNATFTCSFSNTSESFVLNWYRMSPSNQTDKLAAFPEDRSQPGQDSRFRVTQLPNGRDFHMSVVRARRNDSGTYLCGAISLAPKVQIKESLRAELRVTERRAEVPTAHPSPSPRPAGQFQGGGGSGGGGSGGGGSGDIQMTQSPSSLSASVGDRVTITCRASQDVNTAVAWYQQKPGKAPKLLIYSASFLYSGVPSRFSGSRSGTDFTLTISSLQPEDFATYYCQQHYTTPPTFGQGTKVEIKRTVAAPSVFIFPPSDEQLKSGTASVVCLLNNFYPREAKVQWKVDNALQSGNSQESVTEQDSKDSTYSLSSTLTLSKADYEKHKVYACEVTHQGLSSPVTKSFNRGEC

SEQ ID NO: 33 - DNA, 357 bp, Artificial Sequence
  Synthesized
caggtgcagctgcaggagagcggccccggcctggtgaagcccagcgagaccctgagcctgacctgcaccgtgagcggcggcagcgtgagcagcggcgactactactggacctggatccgccagagccccggcaagggcctggagtggatcggccacatctactacagcggcaacaccaactacaaccccagcctgaagagccgcctgaccatcagcatcgacaccagcaagacccagttcagcctgaagctgagcagcgtgaccgccgccgacaccgccatctactactgcgtgcgcgaccgcgtgaccggcgccttcgacatctggggccagggcaccatggtgactgtgtctagc

SEQ ID NO: 34 - protein, 119 aa, Artificial Sequence [sequence omitted]

SEQ ID NO: 35 - DNA, 321 bp, Artificial Sequence
  Synthesized
gacatccagatgacccagagccccagcagcctgagcgccagcgtgggcgaccgcgtgaccatcacctgccaggccagccaggacatcagcaactacctgaactggtaccagcagaagcccggcaaggcccccaagctgctgatctacgacgccagcaacctggagaccggcgtgcccagccgcttcagcggcagcggcagcggcaccgacttcaccttcaccatcagcagcctgcagcccgaggacatcgccacctacttctgccagcacttcgaccacctgcccctggccttcggcggcggcaccaaggtggagatcaag

SEQ ID NO: 36 - protein, 107 aa, Artificial Sequence [sequence omitted]

SEQ ID NO: 37 - DNA, 360 bp, Artificial Sequence
  Synthesized
gaggtgcagctggtggagtctggaggaggcttggtccagcctggggggtccctgagactctcctgtgcagcctctgggttcaatattaaggacacttacatccactgggtccgccaggctccagggaaggggctggagtgggtcgcacgtatttatcctaccaatggttacacacgctacgcagactccgtgaagggccgattcaccatctccgcagacacttccaagaacacggcgtatcttcaaatgaacagcctgagagccgaggacacggccgtgtattactgttcgagatggggcggtgacggcttctatgccatggactactggggccaaggaaccctggtcaccgtctcctca

SEQ ID NO: 38 - protein, 120 aa, Artificial Sequence [sequence omitted]

SEQ ID NO: 39 - DNA, 321 bp, Artificial Sequence
  Synthesized
gacatccagatgacccagtctccatcctccctgtctgcatctgtaggagacagagtcaccatcacttgccgggcaagtcaggatgtgaataccgcggtcgcatggtatcagcagaaaccagggaaagcccctaagctcctgatctattctgcatccttcttgtatagtggggtcccatcaaggttcagtggcagtagatctgggacagatttcactctcaccatcagcagtctgcaacctgaagattttgcaacttactactgtcaacagcattacactacccctccgacgttcggccaaggtaccaaggtggagatcaaa

SEQ ID NO: 40 - protein, 107 aa, Artificial Sequence [sequence omitted]

SEQ ID NO: 41 - DNA, 345 bp, Artificial Sequence
  Synthesized
caggtgcagctggtgcagagcggcgccgaggtgaagaagcccggcgccagcgtgaaggtgagctgcaaggccagcggctacaccttcaccgactacgagatgcactgggtgcgccaggcccccggccagggcctggagtggatgggcgccctggaccccaagaccggcgacaccgcctacagccagaagttcaagggccgcgtgaccctgaccgccgacaagagcaccagcaccgcctacatggagctgagcagcctgaccagcgaggacaccgccgtgtactactgcacccgcttctacagctacacctactggggccagggcaccctggtgaccgtgagcagc

SEQ ID NO: 42 - protein, 115 aa, Artificial Sequence
  Synthesized
QVQLVQSGAEVKKPGASVKVSCKASGYTFTDYEMHWVRQAPGQGLEWMGALDPKTGDTAYSQKFKGRVTLTADKSTSTAYMELSSLTSEDTAVYYCTRFYSYTYWGQGTLVTVSS

SEQ ID NO: 43 - DNA, 336 bp, Artificial Sequence
  Synthesized
gacgtggtgatgacccagagccccctgagcctgcccgtgacccccggcgagcccgccagcatcagctgccgcagcagccagagcctggtgcacagcaaccgcaacacctacctgcactggtacctgcagaagcccggccagagcccccagctgctgatctacaaggtgagcaaccgcttcagcggcgtgcccgaccgcttcagcggcagcggcagcggcaccgacttcaccctgaagatcagccgcgtggaggccgaggacgtgggcgtgtactactgcagccagaacacccacgtgccccccaccttcggccagggcaccaagctggagatcaag

SEQ ID NO: 44 - protein, 112 aa, Artificial Sequence
  Synthesized
DVVMTQSPLSLPVTPGEPASISCRSSQSLVHSNRNTYLHWYLQKPGQSPQLLIYKVSNRFSGVPDRFSGSGSGTDFTLKISRVEAEDVGVYYCSQNTHVPPTFGQGTKLEIK

SEQ ID NO: 45 - protein, 5 aa, Artificial Sequence
  Synthesized
DYEMH

SEQ ID NO: 46 - protein, 17 aa, Artificial Sequence
  Synthesized
ALDPKTGDTAYSQKFKG

SEQ ID NO: 47 - protein, 6 aa, Artificial Sequence
  Synthesized
FYSYTY

SEQ ID NO: 48 - protein, 16 aa, Artificial Sequence
  Synthesized
RSSQSLVHSNRNTYLH

SEQ ID NO: 49 - protein, 7 aa, Artificial Sequence
  Synthesized
KVSNRFS

SEQ ID NO: 50 - protein, 9 aa, Artificial Sequence
  Synthesized
SQNTHVPPT

SEQ ID NO: 51 - DNA, 1809 bp, Artificial Sequence
  Synthesized
ctggacagcccagataggccatggaacccacctactttctctcctgcactgctggtggttacagaaggagataatgctacctttacttgctccttttccaacactagtgagagttttgtccttaattggtatagaatgtctccttcaaatcagacggacaagctcgctgcatttcctgaggaccgcagtcagccggggcaagattccagattccgcgtgacccagctccccaacggacgcgattttcacatgtccgttgtcagggcacgacgcaacgatagtgggacttatctgtgcggggcgatcagtctggccccgaaggtccagataaaagagtccctccgcgctgaactcagggtgaccgagagacgggccgaagtgcccacagcacacccaagtccaagcccaagacctgctgggcaattccaaggtggaggtggatcaggtggcggcggcagtggcgggggcgggagcgggcaggtgcagctggtgcagagcggcgccgaggtgaagaagcccggcgccagcgtgaaggtgagctgcaaggccagcggctacaccttcaccgactacgagatgcactgggtgcgccaggcccccggccagggcctggagtggatgggcgccctggaccccaagaccggcgacaccgcctacagccagaagttcaagggccgcgtgaccctgaccgccgacaagagcaccagcaccgcctacatggagctgagcagcctgaccagcgaggacaccgccgtgtactactgcacccgcttctacagctacacctactggggccagggcaccctggtgaccgtgagcagcgcctccaccaagggcccatcggtcttccccctggcaccctcctccaagagcacctctgggggcacagcggccctgggctgcctggtcaaggactacttccccgaaccggtgacggtgtcgtggaactcaggcgccctgaccagcggcgtgcacaccttcccggctgtcctacagtcctcaggactctactccctcagcagcgtggtgactgtgccctctagcagcttgggcacccagacctacatctgcaacgtgaatcacaagcccagcaacaccaaggtggacaagaaagttgaacccaaatcttgcgacaaaactcacacatgcccaccgtgcccagcacctccagtcgccggaccgtcagtcttcctcttccctccaaaacccaaggacaccctcatgatctcccggacccctgaggtcacatgcgtggtggtggacgtgagccacgaagaccctgaggtcaagttcaactggtacgtggacggcgtggaggtgcataatgccaagacaaagccgcgggaggagcagtacaacagcacgtaccgtgtggtcagcgtcctcaccgtcctgcaccaggactggctgaatggcaaggagtacaagtgcaaggtctccaacaaaggcctcccaagctccatcgagaaaaccatctccaaagccaaagggcagccccgagaaccacaggtgtacaccctgcctccatcccgggatgagctgaccaagaaccaggtcagcctgacctgcctggtcaaaggcttctatcccagcgacatcgccgtggagtgggagagcaatgggcagccggagaacaactacaagaccacgcctcccgtgctggactccgacggctccttcttcctctacagcaagctcaccgtggacaagagcaggtggcagcaggggaacgtcttctcatgctccgtgatgcatgaggctctgcacaaccactacacgcagaagagcctctccctgtctccgggtaaa

SEQ ID NO: 52 - protein, 603 aa, Artificial Sequence
  Synthesized
LDSPDRPWNPPTFSPALLVVTEGDNATFTCSFSNTSESFVLNWYRMSPSNQTDKLAAFPEDRSQPGQDSRFRVTQLPNGRDFHMSVVRARRNDSGTYLCGAISLAPKVQIKESLRAELRVTERRAEVPTAHPSPSPRPAGQFQGGGGSGGGGSGGGGSGQVQLVQSGAEVKKPGASVKVSCKASGYTFTDYEMHWVRQAPGQGLEWMGALDPKTGDTAYSQKFKGRVTLTADKSTSTAYMELSSLTSEDTAVYYCTRFYSYTYWGQGTLVTVSSASTKGPSVFPLAPSSKSTSGGTAALGCLVKDYFPEPVTVSWNSGALTSGVHTFPAVLQSSGLYSLSSVVTVPSSSLGTQTYICNVNHKPSNTKVDKKVEPKSCDKTHTCPPCPAPPVAGPSVFLFPPKPKDTLMISRTPEVTCVVVDVSHEDPEVKFNWYVDGVEVHNAKTKPREEQYNSTYRVVSVLTVLHQDWLNGKEYKCKVSNKGLPSSIEKTISKAKGQPREPQVYTLPPSRDELTKNQVSLTCLVKGFYPSDIAVEWESNGQPENNYKTTPPVLDSDGSFFLYSKLTVDKSRWQQGNVFSCSVMHEALHNHYTQKSLSLSPGK

SEQ ID NO: 53 - DNA, 1134 bp, Artificial Sequence
  Synthesized
ctggacagcccagataggccatggaacccacctactttctctcctgcactgctggtggttacagaaggagataatgctacctttacttgctccttttccaacactagtgagagttttgtccttaattggtatagaatgtctccttcaaatcagacggacaagctcgctgcatttcctgaggaccgcagtcagccggggcaagattccagattccgcgtgacccagctccccaacggacgcgattttcacatgtccgttgtcagggcacgacgcaacgatagtgggacttatctgtgcggggcgatcagtctggccccgaaggtccagataaaagagtccctccgcgctgaactcagggtgaccgagagacgggccgaagtgcccacagcacacccaagtccaagcccaagacctgctgggcaattccaaggcggaggcggatccggaggcggaggttccggcgggggtgggagcggggacgtggtgatgacccagagccccctgagcctgcccgtgacccccggcgagcccgccagcatcagctgccgcagcagccagagcctggtgcacagcaaccgcaacacctacctgcactggtacctgcagaagcccggccagagcccccagctgctgatctacaaggtgagcaaccgcttcagcggcgtgcccgaccgcttcagcggcagcggcagcggcaccgacttcaccctgaagatcagccgcgtggaggccgaggacgtgggcgtgtactactgcagccagaacacccacgtgccccccaccttcggccagggcaccaagctggagatcaagcgcacagtggcagcccccagcgtcttcatttttcccccttccgatgaacagctgaagtccggcactgcttctgtggtctgtctgctgaacaatttctatcccagagaggccaaggtgcagtggaaagtggacaacgctctgcagtccggcaacagccaggagagtgtgaccgaacaggatagtaaggacagcacatattctctgtctagtaccctgacactgagtaaggcagattacgagaagcacaaagtgtatgcctgcgaagtcactcatcagggactgtcaagccccgtgaccaagagcttcaaccggggcgagtgt

SEQ ID NO: 54 - protein, 378 aa, Artificial Sequence
  Synthesized
LDSPDRPWNPPTFSPALLVVTEGDNATFTCSFSNTSESFVLNWYRMSPSNQTDKLAAFPEDRSQPGQDSRFRVTQLPNGRDFHMSVVRARRNDSGTYLCGAISLAPKVQIKESLRAELRVTERRAEVPTAHPSPSPRPAGQFQGGGGSGGGGSGGGGSGDVVMTQSPLSLPVTPGEPASISCRSSQSLVHSNRNTYLHWYLQKPGQSPQLLIYKVSNRFSGVPDRFSGSGSGTDFTLKISRVEAEDVGVYYCSQNTHVPPTFGQGTKLEIKRTVAAPSVFIFPPSDEQLKSGTASVVCLLNNFYPREAKVQWKVDNALQSGNSQESVTEQDSKDSTYSLSSTLTLSKADYEKHKVYACEVTHQGLSSPVTKSFNRGEC

SEQ ID NO: 55 - DNA, 1134 bp, Artificial Sequence
  Synthesized
gacgtggtgatgacccagagccccctgagcctgcccgtgacccccggcgagcccgccagcatcagctgccgcagcagccagagcctggtgcacagcaaccgcaacacctacctgcactggtacctgcagaagcccggccagagcccccagctgctgatctacaaggtgagcaaccgcttcagcggcgtgcccgaccgcttcagcggcagcggcagcggcaccgacttcaccctgaagatcagccgcgtggaggccgaggacgtgggcgtgtactactgcagccagaacacccacgtgccccccaccttcggccagggcaccaagctggagatcaagcgcacagtggcagcccccagcgtcttcatttttcccccttccgatgaacagctgaagtccggcactgcttctgtggtctgtctgctgaacaatttctatcccagagaggccaaggtgcagtggaaagtggacaacgctctgcagtccggcaacagccaggagagtgtgaccgaacaggatagtaaggacagcacatattctctgtctagtaccctgacactgagtaaggcagattacgagaagcacaaagtgtatgcctgcgaagtcactcatcagggactgtcaagccccgtgaccaagagcttcaaccggggcgagtgtggtggaggtggatcaggtggcggcggcagtggcgggggcgggagcgggctggacagcccagataggccatggaacccacctactttctctcctgcactgctggtggttacagaaggagataatgctacctttacttgctccttttccaacactagtgagagttttgtccttaattggtatagaatgtctccttcaaatcagacggacaagctcgctgcatttcctgaggaccgcagtcagccggggcaagattccagattccgcgtgacccagctccccaacggacgcgattttcacatgtccgttgtcagggcacgacgcaacgatagtgggacttatctgtgcggggcgatcagtctggccccgaaggtccagataaaagagtccctccgcgctgaactcagggtgaccgagagacgggccgaagtgcccacagcacacccaagtccaagcccaagacctgctgggcaattccaa

SEQ ID NO: 56 - protein, 378 aa, Artificial Sequence
  Synthesized
DVVMTQSPLSLPVTPGEPASISCRSSQSLVHSNRNTYLHWYLQKPGQSPQLLIYKVSNRFSGVPDRFSGSGSGTDFTLKISRVEAEDVGVYYCSQNTHVPPTFGQGTKLEIKRTVAAPSVFIFPPSDEQLKSGTASVVCLLNNFYPREAKVQWKVDNALQSGNSQESVTEQDSKDSTYSLSSTLTLSKADYEKHKVYACEVTHQGLSSPVTKSFNRGECGGGGSGGGGSGGGGSGLDSPDRPWNPPTFSPALLVVTEGDNATFTCSFSNTSESFVLNWYRMSPSNQTDKLAAFPEDRSQPGQDSRFRVTQLPNGRDFHMSVVRARRNDSGTYLCGAISLAPKVQIKESLRAELRVTERRAEVPTAHPSPSPRPAGQFQ

SEQ ID NO: 57 - DNA, 1332 bp, Artificial Sequence
  Synthesized
caggtgcagctggtgcagagcggcgccgaggtgaagaagcccggcgccagcgtgaaggtgagctgcaaggccagcggctacaccttcaccgactacgagatgcactgggtgcgccaggcccccggccagggcctggagtggatgggcgccctggaccccaagaccggcgacaccgcctacagccagaagttcaagggccgcgtgaccctgaccgccgacaagagcaccagcaccgcctacatggagctgagcagcctgaccagcgaggacaccgccgtgtactactgcacccgcttctacagctacacctactggggccagggcaccctggtgaccgtgagcagcgcctccaccaagggcccatcggtcttccccctggcaccctcctccaagagcacctctgggggcacagcggccctgggctgcctggtcaaggactacttccccgaaccggtgacggtgtcgtggaactcaggcgccctgaccagcggcgtgcacaccttcccggctgtcctacagtcctcaggactctactccctcagcagcgtggtgactgtgccctctagcagcttgggcacccagacctacatctgcaacgtgaatcacaagcccagcaacaccaaggtggacaagaaagttgaacccaaatcttgcgacaaaactcacacatgcccaccgtgcccagcacctccagtcgccggaccgtcagtcttcctcttccctccaaaacccaaggacaccctcatgatctcccggacccctgaggtcacatgcgtggtggtggacgtgagccacgaagaccctgaggtcaagttcaactggtacgtggacggcgtggaggtgcataatgccaagacaaagccgcgggaggagcagtacaacagcacgtaccgtgtggtcagcgtcctcaccgtcctgcaccaggactggctgaatggcaaggagtacaagtgcaaggtctccaacaaaggcctcccaagctccatcgagaaaaccatctccaaagccaaagggcagccccgagaaccacaggtgtacaccctgcctccatcccgggatgagctgaccaagaaccaggtcagcctgacctgcctggtcaaaggcttctatcccagcgacatcgccgtggagtgggagagcaatgggcagccggagaacaactacaagaccacgcctcccgtgctggactccgacggctccttcttcctctacagcaagctcaccgtggacaagagcaggtggcagcaggggaacgtcttctcatgctccgtgatgcatgaggctctgcacaaccactacacgcagaagagcctctccctgtctccgggtaaa

SEQ ID NO: 58 - protein, 444 aa, Artificial Sequence
  Synthesized
QVQLVQSGAEVKKPGASVKVSCKASGYTFTDYEMHWVRQAPGQGLEWMGALDPKTGDTAYSQKFKGRVTLTADKSTSTAYMELSSLTSEDTAVYYCTRFYSYTYWGQGTLVTVSSASTKGPSVFPLAPSSKSTSGGTAALGCLVKDYFPEPVTVSWNSGALTSGVHTFPAVLQSSGLYSLSSVVTVPSSSLGTQTYICNVNHKPSNTKVDKKVEPKSCDKTHTCPPCPAPPVAGPSVFLFPPKPKDTLMISRTPEVTCVVVDVSHEDPEVKFNWYVDGVEVHNAKTKPREEQYNSTYRVVSVLTVLHQDWLNGKEYKCKVSNKGLPSSIEKTISKAKGQPREPQVYTLPPSRDELTKNQVSLTCLVKGFYPSDIAVEWESNGQPENNYKTTPPVLDSDGSFFLYSKLTVDKSRWQQGNVFSCSVMHEALHNHYTQKSLSLSPGK

SEQ ID NO: 59 - DNA, 657 bp, Artificial Sequence
  Synthesized
gacgtggtgatgacccagagccccctgagcctgcccgtgacccccggcgagcccgccagcatcagctgccgcagcagccagagcctggtgcacagcaaccgcaacacctacctgcactggtacctgcagaagcccggccagagcccccagctgctgatctacaaggtgagcaaccgcttcagcggcgtgcccgaccgcttcagcggcagcggcagcggcaccgacttcaccctgaagatcagccgcgtggaggccgaggacgtgggcgtgtactactgcagccagaacacccacgtgccccccaccttcggccagggcaccaagctggagatcaagcgcacagtggcagcccccagcgtcttcatttttcccccttccgatgaacagctgaagtccggcactgcttctgtggtctgtctgctgaacaatttctatcccagagaggccaaggtgcagtggaaagtggacaacgctctgcagtccggcaacagccaggagagtgtgaccgaacaggatagtaaggacagcacatattctctgtctagtaccctgacactgagtaaggcagattacgagaagcacaaagtgtatgcctgcgaagtcactcatcagggactgtcaagccccgtgaccaagagcttcaaccggggcgagtgt

SEQ ID NO: 60 - protein, 219 aa, Artificial Sequence
  Synthesized
DVVMTQSPLSLPVTPGEPASISCRSSQSLVHSNRNTYLHWYLQKPGQSPQLLIYKVSNRFSGVPDRFSGSGSGTDFTLKISRVEAEDVGVYYCSQNTHVPPTFGQGTKLEIKRTVAAPSVFIFPPSDEQLKSGTASVVCLLNNFYPREAKVQWKVDNALQSGNSQESVTEQDSKDSTYSLSSTLTLSKADYEKHKVYACEVTHQGLSSPVTKSFNRGEC

SEQ ID NO: 61 - DNA, 345 bp, Artificial Sequence
  Synthesized
gaggtgcagctggtgcagagcggccccgaggtgaagaagcccggcgccaccgtgaagatcagctgcaagaccagcggctacaccttcaccgagtacaccatccactgggtgaagcaggcccccggcaagggcctggagtggatcggcaacatcaaccccaacaacggcggcaccacctacaaccagaagttcgaggacaaggccaccctgaccgtggacaagagcaccgacaccgcctacatggagctgagcagcctgcgcagcgaggacaccgccgtgtactactgcgccgccggctggaacttcgactactggggccagggcaccctacttacagtaagtagc

SEQ ID NO: 62 - protein, 115 aa, Artificial Sequence
  Synthesized
EVQLVQSGPEVKKPGATVKISCKTSGYTFTEYTIHWVKQAPGKGLEWIGNINPNNGGTTYNQKFEDKATLTVDKSTDTAYMELSSLRSEDTAVYYCAAGWNFDYWGQGTLLTVSS

SEQ ID NO: 63 - DNA, 321 bp, Artificial Sequence
  Synthesized
gacatccagatgacccagagccccagcagcctgagcaccagcgtgggcgaccgcgtgaccctgacctgcaaggccagccaggacgtgggcaccgccgtggactggtaccagcagaagcccggccagagccccaagctgctgatctactgggccagcacccgccacaccggcatccccagccgcttcagcggcagcggcagcggcaccgacttcaccctgaccatcagcagcctgcagcccgaggacttcgccgactactactgccagcagtacaacagctaccccctgaccttcggccccggcaccaaggtggacatcaag

SEQ ID NO: 64 - protein, 107 aa, Artificial Sequence
  Synthesized
DIQMTQSPSSLSTSVGDRVTLTCKASQDVGTAVDWYQQKPGQSPKLLIYWASTRHTGIPSRFSGSGSGTDFTLTISSLQPEDFADYYCQQYNSYPLTFGPGTKVDIK

SEQ ID NO: 65 - protein, 121 aa, Artificial Sequence [sequence omitted]

SEQ ID NO: 66 - protein, 107 aa, Artificial Sequence [sequence omitted]

SEQ ID NO: 67 - protein, 119 aa, Artificial Sequence [sequence omitted]

SEQ ID NO: 68 - protein, 107 aa, Artificial Sequence [sequence omitted]

SEQ ID NO: 69 - protein, 119 aa, Artificial Sequence
  Synthesized
QVQLVESGGGVVQPGRSLRLSCAASGFTFSSYDMHWVRQAPGKGLEWVAVIWYDGSNKYYADSVKGRFTISRDNSKNTLYLQMNSLRAEDTAVYYCARGSGNWGFFDYWGQGTLVTVSS

SEQ ID NO: 70 - protein, 107 aa, Artificial Sequence
  Synthesized
DIQMTQSPSSLSASVGDRVTITCRASQGISRWLAWYQQKPEKAPKSLIYAASSLQSGVPSRFSGSGSGTDFTLTISSLQPEDFATYYCQQYNTYPRTFGQGTKVEIK

SEQ ID NO: 71 - protein, 116 aa, Artificial Sequence [sequence omitted]

SEQ ID NO: 72 - protein, 111 aa, Artificial Sequence [sequence omitted]

SEQ ID NO: 73 - protein, 116 aa, Artificial Sequence
  Synthesized
EVQLVQSGAEVKKPGESLKISCKGSGYSFTGYNMNWVRQMPGKGLEWMGNIDPYYGGTTYNRKFKGQVTISADKSISTAYLQWSSLKASDTAMYYCARSVGPFDSWGQGTLVTVSS

SEQ ID NO: 74 - protein, 107 aa, Artificial Sequence
  Synthesized
EIVLTQSPATLSLSPGERATLSCRASENVYSYLAWYQQKPGQAPRLLIYFAKTLAEGIPARFSGSGSGTDFTLTISSLEPEDFAVYYCQHHSDNPWTFGQGTKVEIK

SEQ ID NO: 75 - protein, 120 aa, Artificial Sequence [sequence omitted]

SEQ ID NO: 76 - protein, 107 aa, Artificial Sequence [sequence omitted]

SEQ ID NO: 77 - protein, 118 aa, Artificial Sequence [sequence omitted]

SEQ ID NO: 78 - protein, 107 aa, Artificial Sequence [sequence omitted]

SEQ ID NO: 79 - protein, 118 aa, Artificial Sequence
  Synthesized
QVQLVESGGGVVQPGRSLRLSCAASGFTFSSFGMHWVRQAPGKGLEWVAYISSGSFTIYYADSVKGRFTISRDNSKNTLYLQMNSLRAEDTAVYYCARMRKGYAMDYWGQGTLVTVSS

SEQ ID NO: 80 - protein, 112 aa, Artificial Sequence
  Synthesized
DVVMTQSPLSLPVTLGQPASISCRSSQIIIHSDGNTYLEWFQQRPGQSPRRLIYKVSNRFSGVPDRFSGSGSGTDFTLKISRVEAEDVGVYYCFQGSHVPHTFGQGTKVEIK

SEQ ID NO: 81 - protein, 120 aa, Artificial Sequence
  Synthesized
QVELVQSGAEVKKPGESLKISCKGSGYSFTSYWIGWVRQAPGKGLEWMGIIDPGDSRTRYSPSFQGQVTISADKSISTAYLQWSSLKASDTAMYYCARGQLYGGTYMDGWGQGTLVTVSS

SEQ ID NO: 82 - protein, 111 aa, Artificial Sequence
  Synthesized
DIALTQPASVSGSPGQSITISCTGTSSDIGGYNSVSWYQQHPGKAPKLMIYGVNNRPSGVSNRFSGSKSGNTASLTISGLQAEDEADYYCSSYDIESATPVFGGGTKLTVL

SEQ ID NO: 83 - protein, 115 aa, Artificial Sequence [sequence omitted]

SEQ ID NO: 84 - protein, 108 aa, Artificial Sequence [sequence omitted]

SEQ ID NO: 85 - protein, 117 aa, Artificial Sequence
  Synthesized
EVQLVESGGGLVQPGGSLRLSCAASGFTFSSYNMNWVRQAPGKGLEWVSYISSSSSTIYYADSVKGRFTISRDNAKNSLSLQMNSLRDEDTAVYYCARAYYYGMDVWGQGTTVTVSS

SEQ ID NO: 86 - protein, 107 aa, Artificial Sequence
  Synthesized
DIQMTQSPSSVSASVGDRVTITCRASQGISGWLAWYQQKPGKAPKFLIYAASTLQSGVPSRFSGSGSGTDFTLTISSLQPEDFATYYCQQANSFPPTFGGGTKVEIK

SEQ ID NO: 87 - protein, 113 aa, Artificial Sequence
  Synthesized
QVQLKESGPDLVAPSQSLSITCTVSGFSLSKFGVNWVRQPPGKGLEWLGVIWGDGSTSYNSGLISRLSISKENSKSQVFLKLNSLQADDTATYYCVKPGGDYWGHGTSVTVSS

SEQ ID NO: 88 - protein, 106 aa, Artificial Sequence
  Synthesized
QVVLTQSPVIMSASPGEKVTMTCSASSSISYMYWYQQKPGTSPKRWIYDTSKLASGVPARFSGSGSGTSYSLTISNMEAGDAATYYCHQRDSYPWTFGGGTNLEIK

SEQ ID NO: 89 - protein, 119 aa, Artificial Sequence
  Synthesized
EVQLVESGGGVVQPGRSLRLSCSASGFTFSGYGLSWVRQAPGKGLEWVAMISSGGSYTYYADSVKGRFAISRDNAKNTLFLQMDSLRPEDTGVYFCARHGDDPAWFAYWGQGTPVTVSS

SEQ ID NO: 90 - protein, 110 aa, Artificial Sequence
  Synthesized
DIQLTQSPSSLSASVGDRVTITCSVSSSISSNNLHWYQQKPGKAPKPWIYGTSNLASGVPSRFSGSGSGTDYTFTISSLQPEDIATYYCQQWSSYPYMYTFGQGTKVEIK

SEQ ID NO: 91 - protein, 119 aa, Artificial Sequence
  Synthesized
DVKLVESGGGLVKLGGSLKLSCAASGFTFSNYYMSWVRQTPEKRLELVAAINSDGGITYYLDTVKGRFTISRDNAKNTLYLQMSSLKSEDTALFYCARHRSGYFSMDYWGQGTSVTVSS

SEQ ID NO: 92 - protein, 107 aa, Artificial Sequence
  Synthesized
DIVMTQSQRFMSTTVGDRVSITCKASQNVVSAVAWYQQKPGQSPKLLIYSASNRYTGVPDRFTGSGSGTDFTLTISNMQSEDLADFFCQQYSNYPWTFGGGTKLEIK

SEQ ID NO: 93 - protein, 117 aa, Artificial Sequence
  Synthesized
QVQLVQSGSELKKPGASVKISCKASGYTFTNYGMNWVRQAPGQGLQWMGWINTDSGESTYAEEFKGRFVFSLDTSVNTAYLQITSLTAEDTGMYFCVRVGYDALDYWGQGTLVTVSS

SEQ ID NO: 94 - protein, 106 aa, Artificial Sequence
  Synthesized
EIVLTQSPSSLSASVGDRVTITCSARSSVSYMHWFQQKPGKAPKLWIYRTSNLASGVPSRFSGSGSGTSYCLTINSLQPEDFATYYCQQRSSFPLTFGGGTKLEIK

SEQ ID NO: 95 - protein, 115 aa, Artificial Sequence
  Synthesized
EVQLVESGGGLVQPGGSLRLSCAASGFTFSSSGMSWVRQAPGKGLEWVSVIASSGSNTYYADSVKGRFTISRDNSKNTLYLQMNSLRAEDTAVYYCARSIFYTTWGQGTLVTVSS

SEQ ID NO: 96 - protein, 108 aa, Artificial Sequence
  Synthesized
DIVLTQSPATLSLSPGERATLSCRASQSVRSNYLAWYQQKPGQAPRLLIYGASSRATGVPARFSGSGSGTDFTLTISSLEPEDFAVYYCQQYSNFPITFGQGTKVEIK

SEQ ID NO: 97 - protein, 118 aa, Artificial Sequence
  Synthesized
EVKLEESGGGLVQPGGSMKLSCAASGFTFSDAWMDWVRQSPEKGLEWVAEIRSKASNHATYYAESVKGRFTISRDDSKSSVYLQMNSLRAEDTGIYYCTRWRRFFDSWGQGTTLTVSS

SEQ ID NO: 98 - protein, 106 aa, Artificial Sequence
  Synthesized
QIVLSQSPAILSASPGEKVTMTCRASSSVSYMHWYQQKPGSSPKPWIYATSNLASGVPVRFSGSGSGTSYSLTISRVEAEDAATYYCQQWSSNPLTFGAGTKLELK

SEQ ID NO: 99 - protein, 119 aa, Artificial Sequence [sequence omitted]

SEQ ID NO: 100 - protein, 111 aa, Artificial Sequence [sequence omitted]